European Patent Specification EP 3 967 755 B1, published March 27, 2024. Title: METHODS OF TREATING TISSUE CALCIFICATION. Applicant: ALEXION PHARMACEUTICALS, INC. Application Divisional of 15871159.8. The sequence listing filed with the application follows.

SEQUENCE LISTING (19 sequences)

SEQ ID NO: 1 - protein, 925 aa, Homo sapiens
MERDGCAGGGSRGGEGGRAPREGPAGNGRDRGRSHAAEAPGDPQAAASLLAPMDVGEEPLEKAARARTAKDPNTYKVLSLVLSVCVLTTILGCIFGLKPSCAKEVKSCKGRCFERTFGNCRCDAACVELGNCCLDYQETCIEPEHIWTCNKFRCGEKRLTRSLCACSDDCKDKGDCCINYSSVCQGEKSWVEEPCESINEPQCPAGFETPPTLLFSLDGFRAEYLHTWGGLLPVISKLKKCGTYTKNMRPVYPTKTFPNHYSIVTGLYPESHGIIDNKMYDPKMNASFSLKSKEKFNPEWYKGEPIWVTAKYQGLKSGTFFWPGSDVEINGIFPDIYKMYNGSVPFEERILAVLQWLQLPKDERPHFYTLYLEEPDSSGHSYGPVSSEVIKALQRVDGMVGMLMDGLKELNLHRCLNLILISDHGMEQGSCKKYIYLNKYLGDVKNIKVIYGPAARLRPSDVPDKYYSFNYEGIARNLSCREPNQHFKPYLKHFLPKRLHFAKSDRIEPLTFYLDPQWQLALNPSERKYCGSGFHGSDNVFSNMQALFVGYGPGFKHGIEADTFENIEVYNLMCDLLNLTPAPNNGTHGSLNHLLKNPVYTPKHPKEVHPLVQCPFTRNPRDNLGCSCNPSILPIEDFQTQFNLTVAEEKIIKHETLPYGRPRVLQKENTICLLSQHQFMSGYSQDILMPLWTSYTVDRNDSFSTEDFSNCLYQDFRIPLSPVHKCSFYKNNTKVSYGFLSPPQLNKNSSGIYSEALLTTNIVPMYQSFQVIWRYFHDTLLRKYAEERNGVNVVSGPVFDFDYDGRCDSLENLRQKRRVIRNQEILIPTHFFIVLTSCKDTSQTPLHCENLDTLAFILPHRTDNSESCVHGKHDSSWVEELLMLHRARITDVEHITGLSFYQQRKEPVSDILKLKTHLPTFSQED

SEQ ID NO: 2 - protein, 827 aa, Artificial Sequence
  Description of Artificial Sequence: Synthetic polypeptide
PSCAKEVKSCKGRCFERTFGNCRCDAACVELGNCCLDYQETCIEPEHIWTCNKFRCGEKRLTRSLCACSDDCKDKGDCCINYSSVCQGEKSWVEEPCESINEPQCPAGFETPPTLLFSLDGFRAEYLHTWGGLLPVISKLKKCGTYTKNMRPVYPTKTFPNHYSIVTGLYPESHGIIDNKMYDPKMNASFSLKSKEKFNPEWYKGEPIWVTAKYQGLKSGTFFWPGSDVEINGIFPDIYKMYNGSVPFEERILAVLQWLQLPKDERPHFYTLYLEEPDSSGHSYGPVSSEVIKALQRVDGMVGMLMDGLKELNLHRCLNLILISDHGMEQGSCKKYIYLNKYLGDVKNIKVIYGPAARLRPSDVPDKYYSFNYEGIARNLSCREPNQHFKPYLKHFLPKRLHFAKSDRIEPLTFYLDPQWQLALNPSERKYCGSGFHGSDNVFSNMQALFVGYGPGFKHGIEADTFENIEVYNLMCDLLNLTPAPNNGTHGSLNHLLKNPVYTPKHPKEVHPLVQCPFTRNPRDNLGCSCNPSILPIEDFQTQFNLTVAEEKIIKHETLPYGRPRVLQKENTICLLSQHQFMSGYSQDILMPLWTSYTVDRNDSFSTEDFSNCLYQDFRIPLSPVHKCSFYKNNTKVSYGFLSPPQLNKNSSGIYSEALLTTNIVPMYQSFQVIWRYFHDTLLRKYAEERNGVNVVSGPVFDFDYDGRCDSLENLRQKRRVIRNQEILIPTHFFIVLTSCKDTSQTPLHCENLDTLAFILPHRTDNSESCVHGKHDSSWVEELLMLHRARITDVEHITGLSFYQQRKEPVSDILKLKTHLPTFSQED

SEQ ID NO: 3 - protein, 1058 aa, Artificial Sequence
  Description of Artificial Sequence: Synthetic polypeptide
PSCAKEVKSCKGRCFERTFGNCRCDAACVELGNCCLDYQETCIEPEHIWTCNKFRCGEKRLTRSLCACSDDCKDKGDCCINYSSVCQGEKSWVEEPCESINEPQCPAGFETPPTLLFSLDGFRAEYLHTWGGLLPVISKLKKCGTYTKNMRPVYPTKTFPNHYSIVTGLYPESHGIIDNKMYDPKMNASFSLKSKEKFNPEWYKGEPIWVTAKYQGLKSGTFFWPGSDVEINGIFPDIYKMYNGSVPFEERILAVLQWLQLPKDERPHFYTLYLEEPDSSGHSYGPVSSEVIKALQRVDGMVGMLMDGLKELNLHRCLNLILISDHGMEQGSCKKYIYLNKYLGDVKNIKVIYGPAARLRPSDVPDKYYSFNYEGIARNLSCREPNQHFKPYLKHFLPKRLHFAKSDRIEPLTFYLDPQWQLALNPSERKYCGSGFHGSDNVFSNMQALFVGYGPGFKHGIEADTFENIEVYNLMCDLLNLTPAPNNGTHGSLNHLLKNPVYTPKHPKEVHPLVQCPFTRNPRDNLGCSCNPSILPIEDFQTQFNLTVAEEKIIKHETLPYGRPRVLQKENTICLLSQHQFMSGYSQDILMPLWTSYTVDRNDSFSTEDFSNCLYQDFRIPLSPVHKCSFYKNNTKVSYGFLSPPQLNKNSSGIYSEALLTTNIVPMYQSFQVIWRYFHDTLLRKYAEERNGVNVVSGPVFDFDYDGRCDSLENLRQKRRVIRNQEILIPTHFFIVLTSCKDTSQTPLHCENLDTLAFILPHRTDNSESCVHGKHDSSWVEELLMLHRARITDVEHITGLSFYQQRKEPVSDILKLKTHLPTFSQEDPKSCDKTHTCPPCPAPEAAGAPSVFLFPPKPKDTLMISRTPEVTCVVVDVSHEDPEVKFNWYVDGVEVHNAKTKPREEQYNSTYRVVSVLTVLHQDWLNGKEYKCKVSNKALPAPIEKTISKAKGQPREPQVYTLPPSREEMTKNQVSLTCLVKGFYPSDIAVEWESNGQPENNYKTTPPVLDSDGSFFLYSKLTVDKSRWQQGNVFSCSVMHEALHNHYTQKSLSLSPGK

SEQ ID NO: 4 - protein, 1068 aa, Artificial Sequence
  Description of Artificial Sequence: Synthetic polypeptide
PSCAKEVKSCKGRCFERTFGNCRCDAACVELGNCCLDYQETCIEPEHIWTCNKFRCGEKRLTRSLCACSDDCKDKGDCCINYSSVCQGEKSWVEEPCESINEPQCPAGFETPPTLLFSLDGFRAEYLHTWGGLLPVISKLKKCGTYTKNMRPVYPTKTFPNHYSIVTGLYPESHGIIDNKMYDPKMNASFSLKSKEKFNPEWYKGEPIWVTAKYQGLKSGTFFWPGSDVEINGIFPDIYKMYNGSVPFEERILAVLQWLQLPKDERPHFYTLYLEEPDSSGHSYGPVSSEVIKALQRVDGMVGMLMDGLKELNLHRCLNLILISDHGMEQGSCKKYIYLNKYLGDVKNIKVIYGPAARLRPSDVPDKYYSFNYEGIARNLSCREPNQHFKPYLKHFLPKRLHFAKSDRIEPLTFYLDPQWQLALNPSERKYCGSGFHGSDNVFSNMQALFVGYGPGFKHGIEADTFENIEVYNLMCDLLNLTPAPNNGTHGSLNHLLKNPVYTPKHPKEVHPLVQCPFTRNPRDNLGCSCNPSILPIEDFQTQFNLTVAEEKIIKHETLPYGRPRVLQKENTICLLSQHQFMSGYSQDILMPLWTSYTVDRNDSFSTEDFSNCLYQDFRIPLSPVHKCSFYKNNTKVSYGFLSPPQLNKNSSGIYSEALLTTNIVPMYQSFQVIWRYFHDTLLRKYAEERNGVNVVSGPVFDFDYDGRCDSLENLRQKRRVIRNQEILIPTHFFIVLTSCKDTSQTPLHCENLDTLAFILPHRTDNSESCVHGKHDSSWVEELLMLHRARITDVEHITGLSFYQQRKEPVSDILKLKTHLPTFSQEDPKSCDKTHTCPPCPAPEAAGAPSVFLFPPKPKDTLMISRTPEVTCVVVDVSHEDPEVKFNWYVDGVEVHNAKTKPREEQYNSTYRVVSVLTVLHQDWLNGKEYKCKVSNKALPAPIEKTISKAKGQPREPQVYTLPPSREEMTKNQVSLTCLVKGFYPSDIAVEWESNGQPENNYKTTPPVLDSDGSFFLYSKLTVDKSRWQQGNVFSCSVMHEALHNHYTQKSLSLSPGKDDDDDDDDDD

SEQ ID NO: 5 - protein, 819 aa, Artificial Sequence
  Description of Artificial Sequence: Synthetic polypeptide
SCKGRCFERTFGNCRCDAACVELGNCCLDYQETCIEPEHIWTCNKFRCGEKRLTRSLCACSDDCKDKGDCCINYSSVCQGEKSWVEEPCESINEPQCPAGFETPPTLLFSLDGFRAEYLHTWGGLLPVISKLKKCGTYTKNMRPVYPTKTFPNHYSIVTGLYPESHGIIDNKMYDPKMNASFSLKSKEKFNPEWYKGEPIWVTAKYQGLKSGTFFWPGSDVEINGIFPDIYKMYNGSVPFEERILAVLQWLQLPKDERPHFYTLYLEEPDSSGHSYGPVSSEVIKALQRVDGMVGMLMDGLKELNLHRCLNLILISDHGMEQGSCKKYIYLNKYLGDVKNIKVIYGPAARLRPSDVPDKYYSFNYEGIARNLSCREPNQHFKPYLKHFLPKRLHFAKSDRIEPLTFYLDPQWQLALNPSERKYCGSGFHGSDNVFSNMQALFVGYGPGFKHGIEADTFENIEVYNLMCDLLNLTPAPNNGTHGSLNHLLKNPVYTPKHPKEVHPLVQCPFTRNPRDNLGCSCNPSILPIEDFQTQFNLTVAEEKIIKHETLPYGRPRVLQKENTICLLSQHQFMSGYSQDILMPLWTSYTVDRNDSFSTEDFSNCLYQDFRIPLSPVHKCSFYKNNTKVSYGFLSPPQLNKNSSGIYSEALLTTNIVPMYQSFQVIWRYFHDTLLRKYAEERNGVNVVSGPVFDFDYDGRCDSLENLRQKRRVIRNQEILIPTHFFIVLTSCKDTSQTPLHCENLDTLAFILPHRTDNSESCVHGKHDSSWVEELLMLHRARITDVEHITGLSFYQQRKEPVSDILKLKTHLPTFSQED

SEQ ID NO: 6 - protein, 739 aa, Artificial Sequence
  Description of Artificial Sequence: Synthetic polypeptide
EKSWVEEPCESINEPQCPAGFETPPTLLFSLDGFRAEYLHTWGGLLPVISKLKKCGTYTKNMRPVYPTKTFPNHYSIVTGLYPESHGIIDNKMYDPKMNASFSLKSKEKFNPEWYKGEPIWVTAKYQGLKSGTFFWPGSDVEINGIFPDIYKMYNGSVPFEERILAVLQWLQLPKDERPHFYTLYLEEPDSSGHSYGPVSSEVIKALQRVDGMVGMLMDGLKELNLHRCLNLILISDHGMEQGSCKKYIYLNKYLGDVKNIKVIYGPAARLRPSDVPDKYYSFNYEGIARNLSCREPNQHFKPYLKHFLPKRLHFAKSDRIEPLTFYLDPQWQLALNPSERKYCGSGFHGSDNVFSNMQALFVGYGPGFKHGIEADTFENIEVYNLMCDLLNLTPAPNNGTHGSLNHLLKNPVYTPKHPKEVHPLVQCPFTRNPRDNLGCSCNPSILPIEDFQTQFNLTVAEEKIIKHETLPYGRPRVLQKENTICLLSQHQFMSGYSQDILMPLWTSYTVDRNDSFSTEDFSNCLYQDFRIPLSPVHKCSFYKNNTKVSYGFLSPPQLNKNSSGIYSEALLTTNIVPMYQSFQVIWRYFHDTLLRKYAEERNGVNVVSGPVFDFDYDGRCDSLENLRQKRRVIRNQEILIPTHFFIVLTSCKDTSQTPLHCENLDTLAFILPHRTDNSESCVHGKHDSSWVEELLMLHRARITDVEHITGLSFYQQRKEPVSDILKLKTHLPTFSQED

SEQ ID NO: 7 - protein, 232 aa, Artificial Sequence
  Description of Artificial Sequence: Synthetic polypeptide
EPKSCDKTHTCPPCPAPELLGGPSVFLFPPKPKDTLMISRTPEVTCVVVDVSHEDPEVKFNWYVDGVEVHNAKTKPREEQYNSTYRVVSVLTVLHQDWLNGKEYKCKVSNKALPAPIEKTISKAKGQPREPQVYTLPPSREEMTKNQVSLTCLVKGFYPSDIAVEWESNGQPENNYKTTPPVLDSDGSFFLYSKLTVDKSRWQQGNVFSCSVMHEALHNHYTQKSLSLSPGK

SEQ ID NO: 8 - protein, 227 aa, Artificial Sequence
  Description of Artificial Sequence: Synthetic polypeptide
DKTHTCPPCPAPELLGGPSVFLFPPKPKDTLMISRTPEVTCVVVDVSHEDPEVKFNWYVDGVEVHNAKTKPREEQYNSTYRVVSVLTVLHQDWLNGKEYKCKVSNKALPAPIEKTISKAKGQPREPQVYTLPPSREEMTKNQVSLTCLVKGFYPSDIAVEWESNGQPENNYKTTPPVLDSDGSFFLYSKLTVDKSRWQQGNVFSCSVMHEALHNHYTQKSLSLSPGK

SEQ ID NO: 9 - protein, 1051 aa, Artificial Sequence
  Description of Artificial Sequence: Synthetic polypeptide
SCKGRCFERTFGNCRCDAACVELGNCCLDYQETCIEPEHIWTCNKFRCGEKRLTRSLCACSDDCKDKGDCCINYSSVCQGEKSWVEEPCESINEPQCPAGFETPPTLLFSLDGFRAEYLHTWGGLLPVISKLKKCGTYTKNMRPVYPTKTFPNHYSIVTGLYPESHGIIDNKMYDPKMNASFSLKSKEKFNPEWYKGEPIWVTAKYQGLKSGTFFWPGSDVEINGIFPDIYKMYNGSVPFEERILAVLQWLQLPKDERPHFYTLYLEEPDSSGHSYGPVSSEVIKALQRVDGMVGMLMDGLKELNLHRCLNLILISDHGMEQGSCKKYIYLNKYLGDVKNIKVIYGPAARLRPSDVPDKYYSFNYEGIARNLSCREPNQHFKPYLKHFLPKRLHFAKSDRIEPLTFYLDPQWQLALNPSERKYCGSGFHGSDNVFSNMQALFVGYGPGFKHGIEADTFENIEVYNLMCDLLNLTPAPNNGTHGSLNHLLKNPVYTPKHPKEVHPLVQCPFTRNPRDNLGCSCNPSILPIEDFQTQFNLTVAEEKIIKHETLPYGRPRVLQKENTICLLSQHQFMSGYSQDILMPLWTSYTVDRNDSFSTEDFSNCLYQDFRIPLSPVHKCSFYKNNTKVSYGFLSPPQLNKNSSGIYSEALLTTNIVPMYQSFQVIWRYFHDTLLRKYAEERNGVNVVSGPVFDFDYDGRCDSLENLRQKRRVIRNQEILIPTHFFIVLTSCKDTSQTPLHCENLDTLAFILPHRTDNSESCVHGKHDSSWVEELLMLHRARITDVEHITGLSFYQQRKEPVSDILKLKTHLPTFSQEDEPKSCDKTHTCPPCPAPELLGGPSVFLFPPKPKDTLMISRTPEVTCVVVDVSHEDPEVKFNWYVDGVEVHNAKTKPREEQYNSTYRVVSVLTVLHQDWLNGKEYKCKVSNKALPAPIEKTISKAKGQPREPQVYTLPPSREEMTKNQVSLTCLVKGFYPSDIAVEWESNGQPENNYKTTPPVLDSDGSFFLYSKLTVDKSRWQQGNVFSCSVMHEALHNHYTQKSLSLSPGK

SEQ ID NO: 10 - protein, 1046 aa, Artificial Sequence
  Description of Artificial Sequence: Synthetic polypeptide
SCKGRCFERTFGNCRCDAACVELGNCCLDYQETCIEPEHIWTCNKFRCGEKRLTRSLCACSDDCKDKGDCCINYSSVCQGEKSWVEEPCESINEPQCPAGFETPPTLLFSLDGFRAEYLHTWGGLLPVISKLKKCGTYTKNMRPVYPTKTFPNHYSIVTGLYPESHGIIDNKMYDPKMNASFSLKSKEKFNPEWYKGEPIWVTAKYQGLKSGTFFWPGSDVEINGIFPDIYKMYNGSVPFEERILAVLQWLQLPKDERPHFYTLYLEEPDSSGHSYGPVSSEVIKALQRVDGMVGMLMDGLKELNLHRCLNLILISDHGMEQGSCKKYIYLNKYLGDVKNIKVIYGPAARLRPSDVPDKYYSFNYEGIARNLSCREPNQHFKPYLKHFLPKRLHFAKSDRIEPLTFYLDPQWQLALNPSERKYCGSGFHGSDNVFSNMQALFVGYGPGFKHGIEADTFENIEVYNLMCDLLNLTPAPNNGTHGSLNHLLKNPVYTPKHPKEVHPLVQCPFTRNPRDNLGCSCNPSILPIEDFQTQFNLTVAEEKIIKHETLPYGRPRVLQKENTICLLSQHQFMSGYSQDILMPLWTSYTVDRNDSFSTEDFSNCLYQDFRIPLSPVHKCSFYKNNTKVSYGFLSPPQLNKNSSGIYSEALLTTNIVPMYQSFQVIWRYFHDTLLRKYAEERNGVNVVSGPVFDFDYDGRCDSLENLRQKRRVIRNQEILIPTHFFIVLTSCKDTSQTPLHCENLDTLAFILPHRTDNSESCVHGKHDSSWVEELLMLHRARITDVEHITGLSFYQQRKEPVSDILKLKTHLPTFSQEDDKTHTCPPCPAPELLGGPSVFLFPPKPKDTLMISRTPEVTCVVVDVSHEDPEVKFNWYVDGVEVHNAKTKPREEQYNSTYRVVSVLTVLHQDWLNGKEYKCKVSNKALPAPIEKTISKAKGQPREPQVYTLPPSREEMTKNQVSLTCLVKGFYPSDIAVEWESNGQPENNYKTTPPVLDSDGSFFLYSKLTVDKSRWQQGNVFSCSVMHEALHNHYTQKSLSLSPGK

SEQ ID NO: 11 - protein, 971 aa, Artificial Sequence
  Description of Artificial Sequence: Synthetic polypeptide
EKSWVEEPCESINEPQCPAGFETPPTLLFSLDGFRAEYLHTWGGLLPVISKLKKCGTYTKNMRPVYPTKTFPNHYSIVTGLYPESHGIIDNKMYDPKMNASFSLKSKEKFNPEWYKGEPIWVTAKYQGLKSGTFFWPGSDVEINGIFPDIYKMYNGSVPFEERILAVLQWLQLPKDERPHFYTLYLEEPDSSGHSYGPVSSEVIKALQRVDGMVGMLMDGLKELNLHRCLNLILISDHGMEQGSCKKYIYLNKYLGDVKNIKVIYGPAARLRPSDVPDKYYSFNYEGIARNLSCREPNQHFKPYLKHFLPKRLHFAKSDRIEPLTFYLDPQWQLALNPSERKYCGSGFHGSDNVFSNMQALFVGYGPGFKHGIEADTFENIEVYNLMCDLLNLTPAPNNGTHGSLNHLLKNPVYTPKHPKEVHPLVQCPFTRNPRDNLGCSCNPSILPIEDFQTQFNLTVAEEKIIKHETLPYGRPRVLQKENTICLLSQHQFMSGYSQDILMPLWTSYTVDRNDSFSTEDFSNCLYQDFRIPLSPVHKCSFYKNNTKVSYGFLSPPQLNKNSSGIYSEALLTTNIVPMYQSFQVIWRYFHDTLLRKYAEERNGVNVVSGPVFDFDYDGRCDSLENLRQKRRVIRNQEILIPTHFFIVLTSCKDTSQTPLHCENLDTLAFILPHRTDNSESCVHGKHDSSWVEELLMLHRARITDVEHITGLSFYQQRKEPVSDILKLKTHLPTFSQEDEPKSCDKTHTCPPCPAPELLGGPSVFLFPPKPKDTLMISRTPEVTCVVVDVSHEDPEVKFNWYVDGVEVHNAKTKPREEQYNSTYRVVSVLTVLHQDWLNGKEYKCKVSNKALPAPIEKTISKAKGQPREPQVYTLPPSREEMTKNQVSLTCLVKGFYPSDIAVEWESNGQPENNYKTTPPVLDSDGSFFLYSKLTVDKSRWQQGNVFSCSVMHEALHNHYTQKSLSLSPGK

SEQ ID NO: 12 - protein, 966 aa, Artificial Sequence
  Description of Artificial Sequence: Synthetic polypeptide
EKSWVEEPCESINEPQCPAGFETPPTLLFSLDGFRAEYLHTWGGLLPVISKLKKCGTYTKNMRPVYPTKTFPNHYSIVTGLYPESHGIIDNKMYDPKMNASFSLKSKEKFNPEWYKGEPIWVTAKYQGLKSGTFFWPGSDVEINGIFPDIYKMYNGSVPFEERILAVLQWLQLPKDERPHFYTLYLEEPDSSGHSYGPVSSEVIKALQRVDGMVGMLMDGLKELNLHRCLNLILISDHGMEQGSCKKYIYLNKYLGDVKNIKVIYGPAARLRPSDVPDKYYSFNYEGIARNLSCREPNQHFKPYLKHFLPKRLHFAKSDRIEPLTFYLDPQWQLALNPSERKYCGSGFHGSDNVFSNMQALFVGYGPGFKHGIEADTFENIEVYNLMCDLLNLTPAPNNGTHGSLNHLLKNPVYTPKHPKEVHPLVQCPFTRNPRDNLGCSCNPSILPIEDFQTQFNLTVAEEKIIKHETLPYGRPRVLQKENTICLLSQHQFMSGYSQDILMPLWTSYTVDRNDSFSTEDFSNCLYQDFRIPLSPVHKCSFYKNNTKVSYGFLSPPQLNKNSSGIYSEALLTTNIVPMYQSFQVIWRYFHDTLLRKYAEERNGVNVVSGPVFDFDYDGRCDSLENLRQKRRVIRNQEILIPTHFFIVLTSCKDTSQTPLHCENLDTLAFILPHRTDNSESCVHGKHDSSWVEELLMLHRARITDVEHITGLSFYQQRKEPVSDILKLKTHLPTFSQEDDKTHTCPPCPAPELLGGPSVFLFPPKPKDTLMISRTPEVTCVVVDVSHEDPEVKFNWYVDGVEVHNAKTKPREEQYNSTYRVVSVLTVLHQDWLNGKEYKCKVSNKALPAPIEKTISKAKGQPREPQVYTLPPSREEMTKNQVSLTCLVKGFYPSDIAVEWESNGQPENNYKTTPPVLDSDGSFFLYSKLTVDKSRWQQGNVFSCSVMHEALHNHYTQKSLSLSPGK

SEQ ID NO: 13 - protein, 15 aa, Homo sapiens
EPKSCDKTHTCPPCP

SEQ ID NO: 14 - protein, 10 aa, Homo sapiens
DKTHTCPPCP

SEQ ID NO: 15 - protein, 14 aa, Homo sapiens
PKSCDKTHTCPPCP

SEQ ID NO: 16 - protein, 15 aa, Artificial Sequence
  Description of Artificial Sequence: Synthetic peptide
GGGGSGGGGSGGGGS

SEQ ID NO: 17 - protein, 6 aa, Artificial Sequence
  Description of Artificial Sequence: Synthetic peptide
PSCAKE

SEQ ID NO: 18 - protein, 10 aa, Artificial Sequence
  Description of Artificial Sequence: Synthetic peptide
DDDDDDDDDD

SEQ ID NO: 19 - protein, 50 aa, Artificial Sequence
  Description of Artificial Sequence: Synthetic polypeptide
  MISC_FEATURE (1)..(50): This sequence may encompass 1-10 repeating "Gly Gly Gly Gly Ser" units wherein some positions may be absent
GGGGSGGGGSGGGGSGGGGSGGGGSGGGGSGGGGSGGGGSGGGGSGGGGS